European Patent Specification EP 3 448 877 B1, published July 16, 2025. Title: Peptides and Nanoparticle Formulations Thereof. Applicant: Bradford University. The sequence listing filed with the application follows.

SEQUENCE LISTING (21 sequences)

SEQ ID NO: 1 - protein, 216 aa, Homo sapiens
MAAQGEPQVQFKLVLVGDGGTGKTTFVKRHLTGEFEKKYVATLGVEVHPLVFHTNRGPIKFNVWDTAGQEKFGGLRDGYYIQAQCAIIMFDVTSRVTYKNVPNWHRDLVRVCENIPIVLCGNKVDIKDRKVKAKSIVFHRKKNLQYYDISAKSNYNFEKPFLWLARKLIGDPNLEFVAMPALAPPEVVMDPALAAQYEHDLEVAQTTALPDEDDDL

SEQ ID NO: 2 - protein, 19 aa, Artificial sequence
  N-terminal sequence of Ran (residues 1 to 19)
MAAQGEPQVQFKLVLVGDG

SEQ ID NO: 3 - protein, 14 aa, Artificial sequence
  Residues 129-142 of Ran
RKVKAKSIVFHRKK

SEQ ID NO: 4 - protein, 20 aa, Artificial sequence
  C-terminal region of Ran (residues 191 to 210)
PALAAQYEHDLEVAQTTALP

SEQ ID NO: 5 - protein, 11 aa, Artificial Sequence
  Synthetic
CAQGEPQVQFK

SEQ ID NO: 6 - protein, 13 aa, Artificial Sequence
  Synthetic
CVDIKDRKVKAKS

SEQ ID NO: 7 - protein, 15 aa, Artificial Sequence
  synthetic
CQYEHDLEVAQTTAL

SEQ ID NO: 8 - protein, 11 aa, Artificial Sequence
  Synthetic
CEQGEPQVQFK

SEQ ID NO: 9 - protein, 11 aa, Artificial Sequence
  Synthetic
CASGEPQVQFK

SEQ ID NO: 10 - protein, 11 aa, Artificial Sequence
  Synthetic
CAQMEPQVQFK

SEQ ID NO: 11 - protein, 11 aa, Artificial Sequence
  Synthetic
CAQGFPQVQFK

SEQ ID NO: 12 - protein, 11 aa, Artificial Sequence
  Synthetic
CAQQRPQVQFK

SEQ ID NO: 13 - protein, 11 aa, Artificial Sequence
  Synthetic
CRQGEPQVQFK

SEQ ID NO: 14 - protein, 10 aa, Artificial Sequence
  Synthetic
CAGEPQVQFK

SEQ ID NO: 15 - protein, 10 aa, Artificial Sequence
  Synthetic
CAQEPQVQFK

SEQ ID NO: 16 - protein, 10 aa, Artificial Sequence
  Synthetic
CAQGPQVQFK

SEQ ID NO: 17 - protein, 9 aa, Artificial Sequence
  Synthetic
CAQPQVQFK

SEQ ID NO: 18 - protein, 9 aa, Artificial Sequence
  Synthetic
CGEPQVQFK

SEQ ID NO: 19 - protein, 10 aa, Artificial Sequence
  Synthetic
AQGEPQVQFK

SEQ ID NO: 20 - protein, 9 aa, Artificial Sequence
  Synthetic
QGEPQVQFK

SEQ ID NO: 21 - protein, 8 aa, Artificial Sequence
  Synthetic
GEPQVQFK